European Patent Application EP 4 170 041 A1, published April 26, 2023. Title: METHOD FOR QUANTITATIVE DETERMINATION OF ETHANOLAMINE PHOSPHORIC ACID, OXIDOREDUCTASE FOR QUANTITATIVE DETERMINATION, COMPOSITION FOR QUANTITATIVE DETERMINATION, KIT FOR QUANTITATIVE DETERMINATION, SENSOR TIP AND SENSOR. Applicant: KIKKOMAN CORPORATION. The sequence listing filed with the application follows.

SEQUENCE LISTING (22 sequences)

SEQ ID NO: 1 - DNA, 1392 bp, Paracoccus denitrificans
atgcaagctattgaaaaacgtgcaggcgccttgccttacgaccctctttatgatcctgttaccgcacgtggactgggtccgcgctccgattatgctccgacctactggatcggcaccgcaggagcacctcccccggatgatggcccggttaccggtgatatggacgcagatgtagttgttattgggagcggttacaccgggctgtcatgcgctttacatctggcaaaaatgcatgggatcaaggcagtggtcttggaggccaatggtgttgcctatggctgctctactcggaatggcggccaggcgcaggtttcatctggccgccttaagagatctcaatggattgaacgctggggtcttgatgtcgcccgtcgtcttcacgccgaagtttgtgagggtttcgatctgttccgtggccttattcgtgatcacgctatcgattgtgatccgcaagacggtgggcattattatatcgcacataaagcaagcgctatgccggccttagagaaggagacagccctgctgcgtgatacttttggatatgacgcccgtatgattagccgtgacgagttgcatgaaaccgttgcgcgtgaccaggaagcacatggtgccatgtgggaagccgatggtgtgggtatacacgcggcaaaattagccttcggttatttacgtgccgcaagagagctgggggcccgtgttcacgtagacagcccggtgcaaggctgggaataccgtaatggtgtgcatcacctgcgcaccccgggcggaactgttcgcgcgcgtcgcgtggcagtggccacagcggcctacgcgccgcgttcattacatcctcgccttcgtgaccgtctgatgcctatcatgagtaacagcatcgtgacacgcgtgcttactccggcggaacttgaagcagtcggtattagaaaactgagtccgctgacggatacacggacactgcgccattattatcggttgttaccagacaatcgcctgcagattggtagtagagcagcgataacgggtcgggacgcggctaatcctgcgcatctggacgcgctgcgcgagggtatggcgcgcaaatttcccgctctgagaggcattgctctggattactcctggtggggttgggtagatgtctcgcacgatatgatgccacgcataacggggttacccgatctgcccggagctttttacgctttagggtatggcggcaacggagtaatgtattcggctatggctggccgccggatggcgcagttggtagcgggggaagctgtcccagatttaccaatttttaacaacgaactgccacacgaaggatggcggacgccatttcgccggctgggacagtggggattgtataaattttatcattatagagatgaaagacggtaa

SEQ ID NO: 2 - DNA, 420 bp, Paracoccus denitrificans
atgccacgtactttgaccgctgccgacttacaggccacattcgacgcatttaacagacacgatattgacggtgtcatgacgcactttgccgatgattgtgtattctataccgtttccggcgaacatgagtacggcaatcgcattgaaggcaaagcggcgatagcgcgtgcattcgaagccgtttggaccaccatgcccgatgtgcaatgggcagaacatacacattttctgagcgaagacggaactcgcggtgttagtcagtggacgtttcgcgcgactaatccggatggatcacgtacggaggtgcagggggtggatctgtttcgtatcgcggatgggcggattgtcgagaaacaagcaattcggaagcagagacctgcaatcccggctgctacagcaccggctcttgccggtaaataa

SEQ ID NO: 3 - DNA, 2031 bp, Lichtheimia corymbifera
atgtcctcttcctcaagcgccacgccaaagcctcatccattagaccctttgtccgcagatgagatccgccgcgcagcagccattatccgcgaaaaacgtgggcaggatacttcttatgtgttcaacagtttaactttgaaggaacctgcgaaacagcaaatgatgttgtacttgggttgggtcaacagttcatcgcagcctaagcccgttacaattgaccgcgaagttttcgcagttcttattgatcgtccaagcggtctggttcacgagatgacagttaacttagataagtcggcggttacctcctggaataaagtggaaggacgccagcccaccattaacatctttgaaatgttagaggcggaacgcgaaatcctgaaggatgagcgtgtcaaggaccaatgtcgccagctgggcatcaccgacatgtcaatggtctatgctgacccgtggggggtaggctatcatgagatcaaaggtaaacgtcttgttcaagcgttgttatacgcacgcacgtcccctgacgacaatcaatacgcgcacccccttgacttcaatcccttatacgatctgaacgctaagaaggtgcttgacatcgtcgtgtccaaacgtcgtaattcctcatttgagcgccctgtgatccccatggcgaatcatcactttctgcccgaacaccttggtgaagaccgtcttcgtaaggatattaagccaatcgaaattacacaaccgcagggcgtatcgttttccattcgtgacggtcatcagcttcattggcagaagtgggacatgcatttgtcattcaactaccgcgaaggccttgttatcaataatcttagctaccgtgatatggactccaccgtccgtccaattatttaccgtatgagccttgctgagatggtcgtgccgtatgctaacccctacaaaccgtacaatcataagatggcgttcgacgtaggagagtacggcttagggaatttaacgaatagccttgagttaggttgtgactgtgttggtaagattggttatttagatgcggtgttgtcggatttaaacggggatccctggcatatccctaatgcaatttgcattcatgaggaggatacggggttgttatttaaacactcggactaccgcacagggaaggcgcactctgctcgtagccgtcgtttggtaatttcacatatcgtgacggcggccaactatgattatggactgtactactacttctaccaggatggtaccatccagtacgaagttaaggcaacgggtgaattgaacacccaggtactggccgaggatgaagacgccgcaccctacggcaccattgtggctcctcaagtcgatgcccagcatcatcaacatttgttctccatgcgtatcgacccaatgttagacggaccgaacaactcggtcgcagaggttgacgtggttgcctccgatcttcccgtcggacaccctcacaattctgtgggaaacagcttttatccagtaactaaagtcttcaacactaccgacgaggccaaaacaatggcgtcagttgagcgtcaccgtacatggaaaatcattaacgaaagtaaaatccatccctatgccaagcagccggttggttttaagatgatggctcatcccaccccgccgcttctgcctaagccagggagcatcgtatatgaacgcgcaatgtttgctagtaagacgttatgggtgacgcctcataacgacaagcagttatatcctggcggtttttattgctatcagtcagagccgtcagaaaaccttgggcttccacaatggacgaaggagacacaaaatgtgcgcgataccgatatcgtctgttggctgaactttggcatcactcatatcccacgcgtagaagactttcctatcatgcctattgaaacttgtggaattatgcttaagccggcgaacttcttcttatgtaatcccgggatcgatattccgccctccacacgtcaatcgaccaagagcgcctatgcgaatgatgcaacttgttgtcgtaaaaacaatttataa

SEQ ID NO: 4 - DNA, 2022 bp, Lichtheimia ramosa
atgtcgtcctcaccgatcaagccgtatcctttagatccattaacagccgatgagattcgccgcgcagcagcccttatccgtgaaacgcgcgggcaggacaccacctatgtgttcaactctctgacactgaaggaaccttcgaagcagcaaatgatgtcttaccttgggtggactaactcgcctagtcaccccaagccggtcactattgaccgcgaagtctttgcggtgttaatcgaccgtccatccgggttggtccatgaaatgaccgtgaacttggataaaaaccaggtgacccgctggaataaggttgaaggtcgccaacctacggtaaatgtattcgagatgttggaggcggaacgcgagattttgaaagacgagcgtgttaaagagcaatgccgccaattggggattaatgatatgagtatggtctttgccgatccctggggtgtaggatatcacgaaattaaaggcaaacgtttggttcaggccttgatgtatgcacgtacctctccggatgacaaccaatacgctcatccactggactttaaccctctgtacgatgtgaacgccaagaaagtaatcgacattatcgtgtcaaaacgtcgcaacagtagtttcgatcgtccagtcattcccatggcaaatcatcatttcttgccggagcatttagggcaagatcgccttcgcaaagacatcaagcctattgagatcactcaacctcagggggtttctttcagcatccgcgatggacaccaattacattggcagaagtgggacatgcatttgtcatttaattaccgtgaaggacttgtgatcaacaacttgagctatcgcgacatggatggcactgtccgccccattatttatcgtatgtcgctttccgagatggttgtgccctatgcgaatccatataagccgtataaccacaaaatggccttcgacgttggtgagtacgggcttggtaaccttacaaactctcttgaattagggtgtgactgcgtcggaaagatttgctatttagacgcgacattgtcggatttgaatggagacccgtggcagattcccaatgcaatctgcatccatgaagaagacacaggacttctgtttaagcacacggattaccgcacgggaaaagcacactcggcgcgttctcgtcgtttggttatctctcatatcgttacggcggcaaattacgactacggtttatattattacttctatcaagacggtaccattcagtatgaagttaaagccaccggcgagttgaacactcaggttcttgcggcagacgaagacgctgctccttacggaactattgtggccccgcaggttgacgctcaacaccatcaacatttgttcagtatgcgtatcgacccaatggtcgatggcccgaataactcagtggcggaagtcgacgttgtggcatctgatcttccggtcgggcacccgcacaattctattggtaacagtttttaccccgtaacgaaagtatttaacacgactgatgaggcaaaaacgatggcctccattgaacgccaccgctcatggaaaattattaacgagaacaaaattcatccctatgcaaagcagcccgtaggtttcaaaatgatggcccaccctacgccgcctcttctgcccaaaccaggttctatcgtctacgaacgcgccatgtttgcgagcaaaacattgtgggttactccatacaacgaggagcaacgttatcccggggggttttattgttaccagtcggaaccttcggagaacttaggactgccacagtggacaaaggaaactcagaatgttcgcgatacggatattgtatgttggttgaattttggcatcacccacatccctcgcgttgaggatttcccaatcatgcctatcgaaacgtgcggcgtaatgctgaagccggtaaatttttttttagggaatcccggcattgacatcccgccctccactcgccaaagcacgaagagtgcgtacgcgacggaagcgacttgctgccgcaaaaataatttataa

SEQ ID NO: 5 - DNA, 2007 bp, Syncephalastrum racemosum
atgaccattgtctctccttcacaccccttagacccgcttacccctagtgaaattcgccacgtagccgaaatcgtacgcgccactcgctctcctgatgataagaccccgcgcgattatattttttccagcatttgcttaaaagaacctcataaggacaagacgttggcatacttgcaatcggtgtccgaagaagctgccgctctgatgcctgaacgtgaagctctggtaattctgatcgatcgcccgtcgggccttgtacacgagattttagtttctatcacagatgagaaggtgaaatctgcaaagacccttaagaatgttcaacctactcagcatgtcttagagatgatcgaagcggaaaagatcatcacgaaggatccttcagttatcgaagaatgtcgcaagttaggcattacggatatgaagaatgtctatgctgatccgtggacggtgggttaccatgctcaatttaagtccagtaaacgtttaatgcaggcccttatgtacatgcgcacctctcccgacgacaaccagtatgcgcatcctttagattttgtaccgatttatgatgttaacgcacaaaaggtcgtcgagattttgcgccaggaaacttcggaagcaagcaagtatgatcgtccgacagttccgttagaaaaccatcagtttttaccagagcacattggcgtggaaaacttacgcaaggacatcaagcccatcgaaattacccaaccggagggggtgtcttttacagtgcgcgggcgtgaaatcgaatggcaaaattggagtatgcatgtcgggttcaactatcgtgaaggagttatcattaacaacgtgtcctataaggacaagggcaatgtgcgtccgttattctaccgcgtgtcggtaagtgaaatggtcgtaccgtacgcacaccccaaggagccgttcaaccataagatggcctttgacgtcggggagtacggtttggggaaccttactaacagccttgagctgggctgtgattgtttgggctcgatttattatatggatggtgtctgtaataatctggatggcgaaccctgggtcatccccaatgcaatttgcatccatgaagaggatacgggtttgttattcaaacacaccgattaccgcactgataaagctcacagcgcacgtagccgccgtttggttatctcgcaaattgtgaccgccgccaactatgattatggcttgtatttctacttctaccaagacggtacgtttcagtacgaggtcaaagctaccggggagctgaacactcaagtttttgcggaagacgaaaacccagcaccttatggtaccgcagtcgctccccaagtcgtaggccagcatcatcaacacttatttatgatgcgcattgacccaatgttagatggtcgtctgaactctgttgcccaggttgatgttttaccctccgagtacccagtcggtcacgtcgagaatccaatcggcaacgcctttagtcctattacgactatttacagtgacacgactgaggcgcaggcacatgggaatttagagtcgtcgcgtacatggaagatcattaacgaatctaaactgcatccatatacaaaagaaccagtaggttacaaacttgtgagtcctaacactcccccgatgcttcccaaacctggatcccttgtctatgaacgcgcaaaattcgctactaaaaccatctgggtaactccctatgaccccgatcagatttatcccgccggattctattgctcacaatcaccgggtgacgattcgatgggattgcctgcatggactaaagaaccacaaagcgtacgtggacgtgacgtagttgtgtggcttaccttcggacttacgcacatcccacgcgtggaagacttccccgttatgcctgtagagacgtgcgggtgggcgctgaaagcgtgtaattttttcttagggaatccagggatcgacattccggcagcacagaaggggacctccaagcgcgtaaatggtgcatgttgtgcgtaa

SEQ ID NO: 6 - DNA, 2052 bp, Syncephalastrum racemosum
atgacagtttctgccgtgattcatcctttggaccccttgtctcccgaggagatccgtcatgcatcagcgattatccgccgcgagcgtagtgccgacaagacaatctttatcttcaacagcatctcgctgcgtgaaccccccaaagaccaggtgcttgcacactttggctgggctgctggcccaaaacctgctcagattgatcgtcaggctttcgtcgtccttatcgatcgcccgtccggcttagtgcatgaaattatcgtgtccttaacgacgtccagcgtggtttcatggaaccgtaaacaaggcgtacaaccaacgctgcacgttcaggagatgcttgaggcagaagaggtgatgttgaaagatgaacgtgtcatcgaggaatgccgcaaattaggaatcgaagatatgagtcttgtgtttgccgacacgtggggagtgggctggcataaaacaaagggcaaacgtcttatgcaggctttgatgtatatgcgtacgagccctgatgataaccagtatgcgcatcccttggactttacaccattatacgatgtcaatgagcaaaaagtcatcgatgtgcttgtcgccaagcgccgtaactcaaagttcgaacgtcccgtcatcccccgtgcggaccaccagtttctgccggaacacctgggggagggcaatttgcgcaaagatattaagcccattgaaattattcaaccagagggtgtcagctttcaaatccgcgggcatgagatcgactggcaaaagtggaaccttcacatcggattcaattatcgcgagggacttgttatcagcaacgttagttacaaagacatggacggcacggtacgtcctgtattctatcgcgtatctctggcagaaatggtagtcccctacgcgaatccttacgaaccctacaaccataagatggccttcgatgtaggagagtacggcctgggcaacttgacgaacagtttagaactgggatgtgattgcgtagggagcatcttctacatggacggggtctgttcggatctgaagggagacgcgtgggtcatccccaatgcgatctgcatccatgaagaggacaccgggttattgttcaagcacacagattttcgcaacaacaaagcgcactcagctcgtagtcgtcgtttggttatttcccatatcgttaccgccgccaattatgattatgggttgtattactatttttaccaggatggtactttccaatacgaagtcaaggccacaggagaacttaacactcacgtcttagcggaggatgagaaccccgctccctacggaacaattgtggcacctcagatcgatgcgcaacaccaccaacacttattttccatgcgcattgatccgatggtagacggaccgactaactcggtggctcaggtagacgtggtagctagcgacttgcctgtcggacaccctgacaacgccgtggggaatgcattctcgccaattaccacaatctatgcgaacacagacgaggcacaagcgcgcgccaatggagagacttcccgttactggaagatcatcaacgaagataaaattcacccatatacacgtgaacctgttggttttaagcttatgtgtccgaacacaccacccatgctgccgaaaccgggatccattgcgtatgagcgtgcagtcttcgcttcgaaaacggtctgggttaccccgtacgacgcagaacaattgttcccaggtggtttctactgttatcagtcggaccccgccgatcgtttaggcctgccggagtggacaaaagggaaaaaggacgtaaagaacaaggacattgtcctgtggttaacgttcgggctgacccacattccgcgtgtggaagactttcccattatgcccgtagaaacctgcggctttatgcttaaaccctgtaacttcttccttgcaaacccaggaattgacatcccggcctccgataagcactcgactaaatcggcgtacgctcatgcgcttacgaatggagccaatgggactgggaacggtagcacaaacggctccagctgctgcaataagaattactaa

SEQ ID NO: 7 - DNA, 2052 bp, Syncephalastrum racemosum
atgacactccccactactatccacccattggatccgctgagtcccgaggaaattcgtcatgttagtgagatcatccgaaaacaacgggccgccgacgaaacaacctatatattcaactccatagcactccgtgaaccgcctaaggaacagatcctcgcgcatttcggttggacagatggacctaaaccagttcagattgatcggcaagcgttcgctgtcctcatagaccgcccttcgggattggtccatgagataattgtgagcatcacgaccgcctccatagtttcctgggagactaaggaaggcgttcagcccactctgcatgtacaagaaatgctggaggcagagcaagtgatgctcaaggatgaacgtgtcatcgaggaatgccgaaaactcggtattgaagatatgtcgatggtattcgctgatacatggggagtgggttggcacaaaaccaagggcaaacgattgatgcaagccctcatgtacatgcgcactagtccagacgacaatcagtatgcccatcccctggatttcacacccctgtatgatgtaaacgagcaaaaagtgatagatgttctggtggcgaaaaggcgaaattcgaaattcgagcgaccagtcattccacgagccgaccgccagttcttgccagagcacctcggagaggaaaatctccgcaaagatataaaaccgattgaaattacccagccccaaggtgtcagtttccagattaggggccacgagatcgactggcaaaagtggaacctgcatgtcggattcaattatcgagaaggcctcgtaattaacaatgtcagttacaaggacatggatggcactgttaggcccatgttctatcgagtgagtctggcagaaatggtcgtcccgtatgcgaacccgtacgagccttacaatcacaagatggcttttgacgtgggtgaatatggactcggtaacctcacaaatagcttggagctcggatgtgattgtgtaggtagtatattttatatggacggagtgtgtagcgacatcaagggtgacgcttgggtaattcccaatgcgatttgcatccacgaagaagacacgggcctcctgttcaagcacactgattttaggaacaataaggcgcatagcgctcgaagccgcaggctggtgatttcccacatcgtcacagcggcaaattacgattatggcctgtactattatttttatcaggacggtacatttcagtacgaagtgaaggcgactggagagctcaacactcacgtattggcggaagacgaagaccctgcaccttacggcactattgttgctcctcaggtagacgcgcagcatcatcaacacctctttagtatgcgtattgatccaatggtagatggacctaccaatagtgtggctcaagtagacgtcgtggccagcgatttgcccgtcggtcatcccgataacgccgtgggtaacgcgttcagtccggttacaacgatttacgcagacactgacgaagcgcgggcacgagctaatggagaaacctcccgctactggaagataattaacgaaactcgcatacatccctacactaaagaaccagtaggtttcaaactcatgtgccctaatacacctccgatgctcccgaaaccgggaagcattgcgtacgaacgcgcagtatttgcctcgaatacagtttgggttactccgtacgatgccgagcaactgtttccgggtggattctactgctatcaaagcgatcccgccgaccgcctgggtctgccggagtggactagggagaagaaggacgtgaaaaacaaggacatagttctgtggctgacgtttggtctcactcatattcccagggttgaggattttccaatcatgccggtagaaacatgtggattcatgctgaagccttgtaatttcttcttggcaaacccgggaattgatatccctgctagcgatcgtcatagtagtaagtccgcatatgcaccggcggttgcaaacggagaatatggcataacaaatggaacgacgaatggctcgtcctgttgcagcaagggacactaa

SEQ ID NO: 8 - protein, 463 aa, Paracoccus denitrificans
MQAIEKRAGALPYDPLYDPVTARGLGPRSDYAPTYWIGTAGAPPPDDGPVTGDMDADVVVIGSGYTGLSCALHLAKMHGIKAVVLEANGVAYGCSTRNGGQAQVSSGRLKRSQWIERWGLDVARRLHAEVCEGFDLFRGLIRDHAIDCDPQDGGHYYIAHKASAMPALEKETALLRDTFGYDARMISRDELHETVARDQEAHGAMWEADGVGIHAAKLAFGYLRAARELGARVHVDSPVQGWEYRNGVHHLRTPGGTVRARRVAVATAAYAPRSLHPRLRDRLMPIMSNSIVTRVLTPAELEAVGIRKLSPLTDTRTLRHYYRLLPDNRLQIGSRAAITGRDAANPAHLDALREGMARKFPALRGIALDYSWWGWVDVSHDMMPRITGLPDLPGAFYALGYGGNGVMYSAMAGRRMAQLVAGEAVPDLPIFNNELPHEGWRTPFRRLGQWGLYKFYHYRDERR

SEQ ID NO: 9 - protein, 638 aa, Arthrobacter globiformis
MTPSTIQTASPFRLASAGEISEVQGILRTAGLLGPEKRIAYLGVLDPARGAGSEAEDRRFRVFIHDVSGARPQEVTVSVTNGTVISAVELDTAATGELPVLEEEFEVVEQLLATDERWLKALAARNLDVSKVRVAPLSAGVFEYAEERGRRILRGLAFVQDFPEDSAWAHPVDGLVAYVDVVSKEVTRVIDTGVFPVPAEHGNYTDPELTGPLRTTQKPISITQPEGPSFTVTGGNHIEWEKWSLDVGFDVREGVVLHNIAFRDGDRLRPIINRASIAEMVVPYGDPSPIRSWQNYFDTGEYLVGQYANSLELGCDCLGDITYLSPVISDAFGNPREIRNGICMHEEDWGILAKHSDLWSGINYTRRNRRMVISFFTTIGNYDYGFYWYLYLDGTIEFEAKATGVVFTSAFPEGGSDNISQLAPGLGAPFHQHIFSARLDMAIDGFTNRVEEEDVVRQTMGPGNERGNAFSRKRTVLTRESEAVREADARTGRTWIISNPESKNRLNEPVGYKLHAHNQPTLLADPGSSIARRAAFATKDLWVTRYADDERYPTGDFVNQHSGGAGLPSYIAQDRDIDGQDIVVWHTFGLTHFPRVEDWPIMPVDTVGFKLRPEGFFDRSPVLDVPANPSQSGSHCHG

SEQ ID NO: 10 - protein, 676 aa, Lichtheimia corymbifera
MSSSSSATPKPHPLDPLSADEIRRAAAIIREKRGQDTSYVFNSLTLKEPAKQQMMLYLGWVNSSSQPKPVTIDREVFAVLIDRPSGLVHEMTVNLDKSAVTSWNKVEGRQPTINIFEMLEAEREILKDERVKDQCRQLGITDMSMVYADPWGVGYHEIKGKRLVQALLYARTSPDDNQYAHPLDFNPLYDLNAKKVLDIVVSKRRNSSFERPVIPMANHHFLPEHLGEDRLRKDIKPIEITQPQGVSFSIRDGHQLHWQKWDMHLSFNYREGLVINNLSYRDMDSTVRPIIYRMSLAEMVVPYANPYKPYNHKMAFDVGEYGLGNLTNSLELGCDCVGKIGYLDAVLSDLNGDPWHIPNAICIHEEDTGLLFKHSDYRTGKAHSARSRRLVISHIVTAANYDYGLYYYFYQDGTIQYEVKATGELNTQVLAEDEDAAPYGTIVAPQVDAQHHQHLFSMRIDPMLDGPNNSVAEVDVVASDLPVGHPHNSVGNSFYPVTKVFNTTDEAKTMASVERHRTWKIINESKIHPYAKQPVGFKMMAHPTPPLLPKPGSIVYERAMFASKTLWVTPHNDKQLYPGGFYCYQSEPSENLGLPQWTKETQNVRDTDIVCWLNFGITHIPRVEDFPIMPIETCGIMLKPANFFLCNPGIDIPPSTRQSTKSAYANDATCCRKNNL

SEQ ID NO: 11 - protein, 673 aa, Lichtheimia ramosa
MSSSPIKPYPLDPLTADEIRRAAALIRETRGQDTTYVFNSLTLKEPSKQQMMSYLGWTNSPSHPKPVTIDREVFAVLIDRPSGLVHEMTVNLDKNQVTRWNKVEGRQPTVNVFEMLEAEREILKDERVKEQCRQLGINDMSMVFADPWGVGYHEIKGKRLVQALMYARTSPDDNQYAHPLDFNPLYDVNAKKVIDIIVSKRRNSSFDRPVIPMANHHFLPEHLGQDRLRKDIKPIEITQPQGVSFSIRDGHQLHWQKWDMHLSFNYREGLVINNLSYRDMDGTVRPIIYRMSLSEMVVPYANPYKPYNHKMAFDVGEYGLGNLTNSLELGCDCVGKICYLDATLSDLNGDPWQIPNAICIHEEDTGLLFKHTDYRTGKAHSARSRRLVISHIVTAANYDYGLYYYFYQDGTIQYEVKATGELNTQVLAADEDAAPYGTIVAPQVDAQHHQHLFSMRIDPMVDGPNNSVAEVDVVASDLPVGHPHNSIGNSFYPVTKVFNTTDEAKTMASIERHRSWKIINENKIHPYAKQPVGFKMMAHPTPPLLPKPGSIVYERAMFASKTLWVTPYNEEQRYPGGFYCYQSEPSENLGLPQWTKETQNVRDTDIVCWLNFGITHIPRVEDFPIMPIETCGVMLKPVNFFLGNPGIDIPPSTRQSTKSAYATEATCCRKNNL

SEQ ID NO: 12 - protein, 668 aa, Syncephalastrum racemosum
MTIVSPSHPLDPLTPSEIRHVAEIVRATRSPDDKTPRDYIFSSICLKEPHKDKTLAYLQSVSEEAAALMPEREALVILIDRPSGLVHEILVSITDEKVKSAKTLKNVQPTQHVLEMIEAEKIITKDPSVIEECRKLGITDMKNVYADPWTVGYHAQFKSSKRLMQALMYMRTSPDDNQYAHPLDFVPIYDVNAQKVVEILRQETSEASKYDRPTVPLENHQFLPEHIGVENLRKDIKPIEITQPEGVSFTVRGREIEWQNWSMHVGFNYREGVIINNVSYKDKGNVRPLFYRVSVSEMVVPYAHPKEPFNHKMAFDVGEYGLGNLTNSLELGCDCLGSIYYMDGVCNNLDGEPWVIPNAICIHEEDTGLLFKHTDYRTDKAHSARSRRLVISQIVTAANYDYGLYFYFYQDGTFQYEVKATGELNTQVFAEDENPAPYGTAVAPQVVGQHHQHLFMMRIDPMLDGRLNSVAQVDVLPSEYPVGHVENPIGNAFSPITTIYSDTTEAQAHGNLESSRTWKIINESKLHPYTKEPVGYKLVSPNTPPMLPKPGSLVYERAKFATKTIWVTPYDPDQIYPAGFYCSQSPGDDSMGLPAWTKEPQSVRGRDVVVWLTFGLTHIPRVEDFPVMPVETCGWALKACNFFLGNPGIDIPAAQKGTSKRVNGACCA

SEQ ID NO: 13 - protein, 683 aa, Syncephalastrum racemosum
MTVSAVIHPLDPLSPEEIRHASAIIRRERSADKTIFIFNSISLREPPKDQVLAHFGWAAGPKPAQIDRQAFVVLIDRPSGLVHEIIVSLTTSSVVSWNRKQGVQPTLHVQEMLEAEEVMLKDERVIEECRKLGIEDMSLVFADTWGVGWHKTKGKRLMQALMYMRTSPDDNQYAHPLDFTPLYDVNEQKVIDVLVAKRRNSKFERPVIPRADHQFLPEHLGEGNLRKDIKPIEIIQPEGVSFQIRGHEIDWQKWNLHIGFNYREGLVISNVSYKDMDGTVRPVFYRVSLAEMVVPYANPYEPYNHKMAFDVGEYGLGNLTNSLELGCDCVGSIFYMDGVCSDLKGDAWVIPNAICIHEEDTGLLFKHTDFRNNKAHSARSRRLVISHIVTAANYDYGLYYYFYQDGTFQYEVKATGELNTHVLAEDENPAPYGTIVAPQIDAQHHQHLFSMRIDPMVDGPTNSVAQVDVVASDLPVGHPDNAVGNAFSPITTIYANTDEAQARANGETSRYWKIINEDKIHPYTREPVGFKLMCPNTPPMLPKPGSIAYERAVFASKTVWVTPYDAEQLFPGGFYCYQSDPADRLGLPEWTKGKKDVKNKDIVLWLTFGLTHIPRVEDFPIMPVETCGFMLKPCNFFLANPGIDIPASDKHSTKSAYAHALTNGANGTGNGSTNGSSCCNKNY

SEQ ID NO: 14 - protein, 683 aa, Syncephalastrum racemosum
MTLPTTIHPLDPLSPEEIRHVSEIIRKQRAADETTYIFNSIALREPPKEQILAHFGWTDGPKPVQIDRQAFAVLIDRPSGLVHEIIVSITTASIVSWETKEGVQPTLHVQEMLEAEQVMLKDERVIEECRKLGIEDMSMVFADTWGVGWHKTKGKRLMQALMYMRTSPDDNQYAHPLDFTPLYDVNEQKVIDVLVAKRRNSKFERPVIPRADRQFLPEHLGEENLRKDIKPIEITQPQGVSFQIRGHEIDWQKWNLHVGFNYREGLVINNVSYKDMDGTVRPMFYRVSLAEMVVPYANPYEPYNHKMAFDVGEYGLGNLTNSLELGCDCVGSIFYMDGVCSDIKGDAWVIPNAICIHEEDTGLLFKHTDFRNNKAHSARSRRLVISHIVTAANYDYGLYYYFYQDGTFQYEVKATGELNTHVLAEDEDPAPYGTIVAPQVDAQHHQHLFSMRIDPMVDGPTNSVAQVDVVASDLPVGHPDNAVGNAFSPVTTIYADTDEARARANGETSRYWKIINETRIHPYTKEPVGFKLMCPNTPPMLPKPGSIAYERAVFASNTVWVTPYDAEQLFPGGFYCYQSDPADRLGLPEWTREKKDVKNKDIVLWLTFGLTHIPRVEDFPIMPVETCGFMLKPCNFFLANPGIDIPASDRHSSKSAYAPAVANGEYGITNGTTNGSSCCSKGH

SEQ ID NO: 15 - DNA, 15 bp, Artificial Sequence
  pKK223-3
caggaaacagaattc

SEQ ID NO: 16 - DNA, 678 bp, Lichtheimia ramosa
atgtcgtcctcaccgatcaagccgtatcctttagatccattaacagccgatgagattcgccgcgcagcagcccttatccgtgaaacgcgcgggcaggacaccacctatgtgttcaactctctgacactgaaggaaccttcgaagcagcaaatgatgtcttaccttgggtggactaactcgcctagtcaccccaagccggtcactattgaccgcgaagtctttgcggtgttaatcgaccgtccatccgggttggtccatgaaatgaccgtgaacttggataaaaaccaggtgacccgctggaataaggttgaaggtcgccaacctacggtaaatgtattcgagatgttggaggcggaacgcgagattttgaaagacgagcgtgttaaagagcaatgccgccaattggggattaatgatatgagtatggtctttgccgatccctggggtgtaggatatcacgaaattaaaggcaaacgtttggttcaggccttgatgtatgcacgtacctctccggatgacaaccaatacgctcatccactggactttaaccctctgtacgatgtgaacgccaagaaagtaatcgacattatcgtgtcaaaacgtcgcaacagtagtttcgatcgtccagtcattcccatggcaaatcatcatttcttgccggagcatttagggcaagat

SEQ ID NO: 17 - DNA, 693 bp, Lichtheimia ramosa
catttagggcaagatcgccttcgcaaagacatcaagcctattgagatcactcaacctcagggggtttctttcagcatccgcgatggacaccaattacattggcagaagtgggacatgcatttgtcatttaattaccgtgaaggacttgtgatcaacaacttgagctatcgcgacatggatggcactgtccgccccattatttatcgtatgtcgctttccgagatggttgtgccctatgcgaatccatataagccgtataaccacaaaatggccttcgacgttggtgagtacgggcttggtaaccttacaaactctcttgaattagggtgtgactgcgtcggaaagatttgctatttagacgcgacattgtcggatttgaatggagacccgtggcagattcccaatgcaatctgcatccatgaagaagacacaggacttctgtttaagcacacggattaccgcacgggaaaagcacactcggcgcgttctcgtcgtttggttatctctcatatcgttacggcggcaaattacgactacggtttatattattacttctatcaagacggtaccattcagtatgaagttaaagccaccggcgagttgaacactcaggttcttgcggcagacgaagacgctgctccttacggaactattgtggccccgcaggttgacgctcaacaccatcaacatttg

SEQ ID NO: 18 - DNA, 681 bp, Lichtheimia ramosa
caccatcaacatttgttcagtatgcgtatcgacccaatggtcgatggcccgaataactcagtggcggaagtcgacgttgtggcatctgatcttccggtcgggcacccgcacaattctattggtaacagtttttaccccgtaacgaaagtatttaacacgactgatgaggcaaaaacgatggcctccattgaacgccaccgctcatggaaaattattaacgagaacaaaattcatccctatgcaaagcagcccgtaggtttcaaaatgatggcccaccctacgccgcctcttctgcccaaaccaggttctatcgtctacgaacgcgccatgtttgcgagcaaaacattgtgggttactccatacaacgaggagcaacgttatcccggggggttttattgttaccagtcggaaccttcggagaacttaggactgccacagtggacaaaggaaactcagaatgttcgcgatacggatattgtatgttggttgaattttggcatcacccacatccctcgcgttgaggatttcccaatcatgcctatcgaaacgtgcggcgtaatgctgaagccggtaaatttttttttagggaatcccggcattgacatcccgccctccactcgccaaagcacgaagagtgcgtacgcgacggaagcgacttgctgccgcaaaaataatttataa

SEQ ID NO: 19 - DNA, 15 bp, Artificial Sequence
  pKK223-3
aagcttggctgtttt

SEQ ID NO: 20 - DNA, 1914 bp, Arthrobacter globiformis
atgacaccgtcaacgattcaaactgccagtccatttcgtttagcatcggctggcgagatcagcgaagtacaaggaatcctgcgcactgcaggcttattgggtcccgagaaacgcattgcttacttgggggtccttgatcctgctcgtggggccggcagcgaagcggaagatcgccgtttccgcgtttttatccacgatgtctcgggagcgcgccctcaagaagtgactgtgtcggtaacgaacggtacggtcatttccgccgtcgaattggatacagccgccactggtgaattaccggtattggaagaagagttcgaggttgtagaacaactgctggcaacggatgagcgttggttaaaggcacttgcggctcgtaaccttgatgttagtaaagtacgcgtagctcctctttctgctggtgtctttgagtacgccgaagaacgcggccgtcgcatccttcgtggcttggcttttgtacaggacttcccagaagattcggcttgggcacatcccgtggacgggcttgtggcctacgttgacgtggtatcaaaggaagtcacccgtgtaattgatactggggttttccccgtaccggcggaacatgggaactacacagatcccgagttgacaggtcctcttcgcacgacacagaagcctatcagcattacacagcccgaaggtccttcatttacggtgacgggcggcaaccatatcgagtgggagaaatggtccctggacgtcggattcgacgttcgtgagggtgtggtgcttcataacattgcttttcgtgacggagatcgccttcgcccgattatcaaccgcgcgtccattgctgaaatggtcgtcccttacggggatccttctcccattcgctcgtggcagaactatttcgatacgggggagtacttagtcggccagtacgccaactcattggaacttggctgtgattgtcttggagatatcacgtacctgtcccctgttatctcagatgcgttcggaaaccctcgtgaaatccgcaacgggatctgtatgcatgaagaagattgggggattcttgcaaaacattcggatttatggtccggcatcaactatacgcgtcgcaatcgtcgtatggtgatttcatttttcacaaccatcgggaattatgattatgggttttattggtatctgtacctggacggaacgatcgagtttgaagcaaaggcaactggagtggtattcacgtctgcgtttcccgagggcgggtccgataatattagccagcttgccccaggccttggcgctccgtttcatcaacacatcttctcggcccgtttagacatggctatcgatggattcacgaatcgtgttgaggaagaggatgttgtgcgccaaacgatgggacccggcaacgaacgtgggaatgcgttcagtcgtaaacgtacggttctgacgcgcgaatcagaagcggtacgtgaggcagacgcacgtacaggtcgcacctggatcatctcaaatcccgagtctaagaatcgtcttaatgaacccgtagggtataagttacacgcccacaaccaaccgaccttactggcggaccctggaagctcaatcgctcgtcgcgcggccttcgccaccaaagatctgtgggtaacacgttacgccgacgatgagcgctatcccacaggagacttcgtaaaccagcattccgggggcgcgggtttgccatcctatattgcccaggaccgcgacatcgatggccaagacatcgtagtatggcatacatttggacttacccactttccacgtgtggaggactggccaattatgccggtggacactgtaggtttcaagcttcgcccagaaggattctttgaccgcagtcctgtgctggatgtaccagccaatccctcccaatctggttcacactgccatgga

SEQ ID NO: 21 - DNA, 975 bp, Arthrobacter globiformis
atgacaccgtcaacgattcaaactgccagtccatttcgtttagcatcggctggcgagatcagcgaagtacaaggaatcctgcgcactgcaggcttattgggtcccgagaaacgcattgcttacttgggggtccttgatcctgctcgtggggccggcagcgaagcggaagatcgccgtttccgcgtttttatccacgatgtctcgggagcgcgccctcaagaagtgactgtgtcggtaacgaacggtacggtcatttccgccgtcgaattggatacagccgccactggtgaattaccggtattggaagaagagttcgaggttgtagaacaactgctggcaacggatgagcgttggttaaaggcacttgcggctcgtaaccttgatgttagtaaagtacgcgtagctcctctttctgctggtgtctttgagtacgccgaagaacgcggccgtcgcatccttcgtggcttggcttttgtacaggacttcccagaagattcggcttgggcacatcccgtggacgggcttgtggcctacgttgacgtggtatcaaaggaagtcacccgtgtaattgatactggggttttccccgtaccggcggaacatgggaactacacagatcccgagttgacaggtcctcttcgcacgacacagaagcctatcagcattacacagcccgaaggtccttcatttacggtgacgggcggcaaccatatcgagtgggagaaatggtccctggacgtcggattcgacgttcgtgagggtgtggtgcttcataacattgcttttcgtgacggagatcgccttcgcccgattatcaaccgcgcgtccattgctgaaatggtcgtcccttacggggatccttctcccattcgctcgtggcagaactatttcgatacgggggagtacttagtcggccagtacgccaactcattggaacttggctgtgattgtcttggagatatcacgtacctgtcc

SEQ ID NO: 22 - DNA, 957 bp, Arthrobacter globiformis
atcacgtacctgtcccctgttatctcagatgcgttcggaaaccctcgtgaaatccgcaacgggatctgtatgcatgaagaagattgggggattcttgcaaaacattcggatttatggtccggcatcaactatacgcgtcgcaatcgtcgtatggtgatttcatttttcacaaccatcgggaattatgattatgggttttattggtatctgtacctggacggaacgatcgagtttgaagcaaaggcaactggagtggtattcacgtctgcgtttcccgagggcgggtccgataatattagccagcttgccccaggccttggcgctccgtttcatcaacacatcttctcggcccgtttagacatggctatcgatggattcacgaatcgtgttgaggaagaggatgttgtgcgccaaacgatgggacccggcaacgaacgtgggaatgcgttcagtcgtaaacgtacggttctgacgcgcgaatcagaagcggtacgtgaggcagacgcacgtacaggtcgcacctggatcatctcaaatcccgagtctaagaatcgtcttaatgaacccgtagggtataagttacacgcccacaaccaaccgaccttactggcggaccctggaagctcaatcgctcgtcgcgcggccttcgccaccaaagatctgtgggtaacacgttacgccgacgatgagcgctatcccacaggagacttcgtaaaccagcattccgggggcgcgggtttgccatcctatattgcccaggaccgcgacatcgatggccaagacatcgtagtatggcatacatttggacttacccactttccacgtgtggaggactggccaattatgccggtggacactgtaggtttcaagcttcgcccagaaggattctttgaccgcagtcctgtgctggatgtaccagccaatccctcccaatctggttcacactgccatggataa